European Patent Application EP 4 807 362 A1, published September 16, 2026. Title: NANOPORE-BASED ANALYSIS OF ANALYTES. Applicant: RIJKSUNIVERSITEIT GRONINGEN. Application NL PCT/NL2023/050570, filed October 30, 2023. The sequence listing filed with the application follows.

SEQUENCE LISTING (58 sequences)

SEQ ID NO: 1 - protein, 15 aa, synthetic construct
GGGGSGGGGSGGGGS

SEQ ID NO: 2 - protein, 5 aa, synthetic construct
GGGGS

SEQ ID NO: 3 - protein, 8 aa, synthetic construct
GGGGGGGG

SEQ ID NO: 4 - protein, 6 aa, synthetic construct
GGGGGG

SEQ ID NO: 5 - protein, 15 aa, synthetic construct
EAAAKEAAAKEAAAK

SEQ ID NO: 6 - protein, 5 aa, synthetic construct
EAAAK

SEQ ID NO: 7 - protein, 17 aa, synthetic construct
VSQTSKLTRAETVFPDV

SEQ ID NO: 8 - protein, 6 aa, synthetic construct
PLGLWA

SEQ ID NO: 9 - protein, 6 aa, synthetic construct
RVLAEA

SEQ ID NO: 10 - protein, 10 aa, synthetic construct
EDVVCCSNSY

SEQ ID NO: 11 - protein, 8 aa, synthetic construct
GGIEGRGS

SEQ ID NO: 12 - protein, 10 aa, synthetic construct
TRHRQPRGWE

SEQ ID NO: 13 - protein, 10 aa, synthetic construct
AGNRVRRSVG

SEQ ID NO: 14 - protein, 9 aa, synthetic construct
RRRRRRRRR

SEQ ID NO: 15 - protein, 4 aa, synthetic construct
GFLG

SEQ ID NO: 16 - protein, 46 aa, synthetic construct
AEAAAKEAAAKEAAAKEAAAKALEAEAAAKEAAAKEAAAKEAAAKA

SEQ ID NO: 17 - protein, 5 aa, synthetic construct
PAPAP

SEQ ID NO: 18 - protein, 12 aa, synthetic construct
AEAAAKEAAAKA

SEQ ID NO: 19 - protein, 11 aa, synthetic construct
AANDENYALAA

SEQ ID NO: 20 - protein, 64 aa, synthetic construct
MAQEQTKRGGGGGDDDDIAGSTAAGQERREKLTEETDDLLDEIDDVLEENAEDFVRAYVQKGGQ

SEQ ID NO: 21 - protein, 21 aa, synthetic construct
SASSHATRQLSGLKIHSNLYH

SEQ ID NO: 22 - protein, 56 aa, synthetic construct
AKSKGKQRGVKQKIHHFHEPMLHNSSEEQVKVEDAFNQRTSTDSRLQSTGTAPRKK

SEQ ID NO: 23 - protein, 267 aa, synthetic construct
SEVFQECVNLFIKRDIKDCLEKMSEVGFIDITVFKSNPMILDLFVSACDIMPSFTKLGLTLQSEILNIFTLDTPQCIETRKIILGDLSKLLVINKFFRCCIKVIQFNLTDHTEQEEKTLELESIMSDFIFVYITKMRTTIDVVGLQELIEIFIFQVKVKLHHKKPSPNMYWALCKTLPKLSPTLKGLYLSKDVSIEDAILNSIDNKIQKDKAKSKGKQRGVKQKIHHFHEPMLHNSSEEQVKVEDAFNQRTSTDSRLQSTGTAPRKK

SEQ ID NO: 24 - protein, 309 aa, synthetic construct
MAASEIMNNLPMHSLDSSLRDLLNDDLFIESDESTKSVNDQRSEVFQECVNLFIKRDIKDCLEKMSEVGFIDITVFKSNPMILDLFVSACDIMPSFTKLGLTLQSEILNIFTLDTPQCIETRKIILGDLSKLLVINKFFRCCIKVIQFNLTDHTEQEEKTLELESIMSDFIFVYITKMRTTIDVVGLQELIEIFIFQVKVKLHHKKPSPNMYWALCKTLPKLSPTLKGLYLSKDVSIEDAILNSIDNKIQKDKAKSKGKQRGVKQKIHHFHEPMLHNSSEEQVKVEDAFNQRTSTDSRLQSTGTAPRKK

SEQ ID NO: 25 - protein, 250 aa, synthetic construct
MGHHHHHHSSASKGEELFTGVVPILVELDGDVNGHKFSVSGEGEGDATYGKLTLKFICTTGKLPVPWPTLVTTFSYGVQCFSRYPDHMKRHDFFKSAMPEGYVQERTIFFKDDGNYKTRAEVKFEGDTLVNRIELKGIDFKEDGNILGHKLEYNYNSHNVYIMADKQKNGIKVNFKIRHNIEDGSVQLADHYQQNTPIGDGPVLLPDNHYLSTQSALSKDPNEKRDHMVLLEFVTAAGIAANDENYALAA

SEQ ID NO: 26 - protein, 278 aa, synthetic construct
MGHHHHHHSSASKGEELFTGVVPILVELDGDVNGHKFSVSGEGEGDATYGKLTLKFICTTGKLPVPWPTLVTTFSYGVQCFSRYPDHMKRHDFFKSAMPEGYVQERTIFFKDDGNYKTRAEVKFEGDTLVNRIELKGIDFKEDGNILGHKLEYNYNSHNVYIMADKQKNGIKVNFKIRHNIEDGSVQLADHYQQNTPIGDGPVLLPDNHYLSTQSALSKDPNEKRDHMVLLEFVTAAGIGGGGGGGGGGGGSRRRRRRRRRRRRRRRAANDENYALAA

SEQ ID NO: 27 - protein, 255 aa, synthetic construct
MGHHHHHHSSASKGEELFTGVVPILVELDGDVNGHKFSVSGEGEGDATYGKLTLKFICTTGKLPVPWPTLVTTFSYGVQCFSRYPDHMKRHDFFKSAMPEGYVQERTIFFKDDGNYKTRAEVKFEGDTLVNRIELKGIDFKEDGNILGHKLEYNYNSHNVYIMADKQKNGIKVNFKIRHNIEDGSVQLADHYQQNTPIGDGPVLLPDNHYLSTQSALSKDPNEKRDHMVLLEFVTAAGIRRRRRAANDENYALAA

SEQ ID NO: 28 - protein, 262 aa, synthetic construct
MGHHHHHHSSASKGEELFTGVVPILVELDGDVNGHKFSVSGEGEGDATYGKLTLKFICTTGKLPVPWPTLVTTFSYGVQCFSRYPDHMKRHDFFKSAMPEGYVQERTIFFKDDGNYKTRAEVKFEGDTLVNRIELKGIDFKEDGNILGHKLEYNYNSHNVYIMADKQKNGIKVNFKIRHNIEDGSVQLADHYQQNTPIGDGPVLLPDNHYLSTQSALSKDPNEKRDHMVLLEFVTAAGIGEGDGEGDGEGDAANDENYALAA

SEQ ID NO: 29 - protein, 422 aa, synthetic construct
MHHHHHHSSPWKIEEGKLVIWINGDKGYNGLAEVGKKFEKDTGIKVTVEHPDKLEEKFPQVAATGDGPDIIFWAHDRFGGYAQSGLLAEITPDKAFQDKLYPFTWDAVRYNGKLIAYPIAVEALSLIYNKDLLPNPPKTWEEIPALDKELKAKGKSALMFNLQEPYFTWPLIAADGGYAFKYENGKYDIKDVGVDNAGAKAGLTFLVDLIKNKHMNADTDYSIAEAAFNKGETAMTINGPWAWSNIDTSKVNYGVTVLPTFKGQPSKPFVGVLSAGINAASPNKELAKEFLENYLLTDEGLEAVNKDKPLGAVALKSYEEELAKDPRIAATMENAQKGEIMPNIPQMSAFWYAVRTAVINAASGRQTVDEALKDAQTRITKHMGGGGGGGGGGGGSRRRRRRRRRRRRRRRAANDENYALAA

SEQ ID NO: 30 - protein, 419 aa, synthetic construct
MHHHHHHSSPWGAPKIEEGKLVIWINGDKGYNGLAEVGKKFEKDTGIKVTVEHPDKLEEKFPQVAATGDGPDIIFWAHDRFGGYAQSGLLAEITPDKAFQDKLYPFTWDAVRYNGKLIAYPIAVEALSLIYNKDLLPNPPKTWEEIPALDKELKAKGKSALMFNLQEPYFTWPLIAADGGYAFKYENGKYDIKDVGVDNAGAKAGLTFLVDLIKNKHMNADTDYSIAEAAFNKGETAMTINGPWAWSNIDTSKVNYGVTVLPTFKGQPSKPFVGVLSAGINAASPNKELAKEFLENYLLTDEGLEAVNKDKPLGAVALKSYEEELAKDPRIAATMENAQKGEIMPNIPQMSAFWYAVRTAVINAASGRQTVDEALKDAQTRITKHMGGGGGGSRRRRRRRRRRRRRRRAANDENYALAA

SEQ ID NO: 31 - protein, 420 aa, synthetic construct
MHHHHHHSSPWGAPKIEEGKLVIWINGDKGYNGLAEVGKKFEKDTGIKVTVEHPDKLEEKFPQVAATGDGPDIIFWAHDRFGGYAQSGLLAEITPDKAFQDKLYPFTWDAVRYNGKLIAYPIAVEALSLIYNKDLLPNPPKTWEEIPALDKELKAKGKSALMFNLQEPYFTWPLIAADGGYAFKYENGKYDIKDVGVDNAGAKAGLTFLVDLIKNKHMNADTDYSIAEAAFNKGETAMTINGPWAWSNIDTSKVNYGVTVLPTFKGQPSKPFVGVLSAGINAASPNKELAKEFLENYLLTDEGLEAVNKDKPLGAVALKSYEEELAKDPRIAATMENAQKGEIMPNIPQMSAFWYAVRTAVINAASGRQTVDEALKDAQTRITKHMGGGGGGGGGGGGGSDDDDDDDDDDAANDENYALA

SEQ ID NO: 32 - protein, 6 aa, synthetic construct
HHHHHH

SEQ ID NO: 33 - protein, 310 aa, synthetic construct
MADSDINIKTGTTDIGSNTTVKTGDLVTYDKENGMHKKVFYSFIDDKNHNKKLLVIRTKGTIAGQYRVYSEEGANKSGLAWPSAFKVQLQLPDNEVAQISDYYPRNSIDTKEYMSTLTYGFNGNVTGDDTGKIGGLIGANVSIGHTLKYVQPDFKTILESPTDKKVGWKVIFNNMVNQNWGPYDRDSWNPVYGNQLFMKTRNGSMKAADNFLDPNKASSLLSSGFSPDFATVITMDRKASKQQTNIDVIYERVRDDYQLHWTSTNWKGTNTKDKWTDRSSERYKIDWEKEEMTNRGSGSSGGSSHHHHHH

SEQ ID NO: 34 - protein, 316 aa, synthetic construct
MAQTTSQVVTDIGQNAKTHTSYNTFNNEQADNMTMSLKVTFIDDPSADKQIAVINTTGSFMKANPTLSDAPVDGYPIPGASVTLRYPSQYDIAMNLQDNTSRFFHVAPTNAVEETTVTSSVSYQLGGSIKASVTPSGPSGESGATGQVTWSDSVSYKQTSYKTNLIDQTNKHVKWNVFFNGYNNQNWGIYTRDSYHALYGNQLFMYSRTYPHETDARGNLVPMNDLPTLTNSGFSPGMIAVVISEKDTEQSSIQVAYTKHADDYTLRPGFTFGTGNWVGNNIKDVDQKTFNKSFVLDWKNKKLVEKKGSAHHHHHH

SEQ ID NO: 35 - protein, 316 aa, synthetic construct
MAQTTSQVVTDIGQNAKTHTSYNTFNNEQADNMTMSLKVTFIDDPSADKQIAVINTTGSFMKANPTLSDAPVDGYPIPGASVTLRYPSQYDIAMNLQDNTSRFFHVAPTNAVEETTVTSSVDYDLGGSIDASVTPSGPSGESGATGQVTWSDSVSYDQTSYKTNLIDQTNKHVKWNVFFNGYNNQNWGIYTRDSYHALYGNQLFMYSRTYPHETDARGNLVPMNDLPTLTNSGFSPGMIAVVISEKDTEQSSIQVAYTKHADDYTLRPGFTFGTGNWVGNNIKDVDQKTFNKSFVLDWKNKKLVEKKGSAHHHHHH

SEQ ID NO: 36 - protein, 316 aa, synthetic construct
MAQTTSQVVTDIGQNAKTHTSYNTFNNEQADNMTMSLKVTFIDDPSADKQIAVINTTGSFMKANPTLSDAPVDGYPIPGASVTLRYPSQYDIAMNLQDNTSRFFHVAPTNAVEETTVTSSVDYQLGGSIDASVTPSGPSGESGATGQVDWSDSVSYDQTSYKTNLIDQTNKHVKWNVFFNGYNNQNWGIYTRDSYHALYGNQLFMYSRTYPHETDARGNLVPMNDLPTLTNSGFSPGMIAVVISEKDTEQSSIQVAYTKHADDYTLRPGFTFGTGNWVGNNIKDVDQKTFNKSFVLDWKNKKLVEKKGSAHHHHHH

SEQ ID NO: 37 - protein, 316 aa, synthetic construct
MAQTTSQVVTDIGQNAKTHTSYNTFNNEQADNMTMSLKVTFIDDPSADKQIAVINTTGSFMKANPTLSDAPVDGYPIPGASVTLRYPSQYDIAMNLQDNTSRFFHVAPTNAVEETTVTSSVDYQLGGSIDASVTPSGPSGESGATGQVTWSDDVSYDQTSYKTNLIDQTNKHVKWNVFFNGYNNQNWGIYTRDSYHALYGNQLFMYSRTYPHETDARGNLVPMNDLPTLTNSGFSPGMIAVVISEKDTEQSSIQVAYTKHADDYTLRPGFTFGTGNWVGNNIKDVDQKTFNKSFVLDWKNKKLVEKKGSAHHHHHH

SEQ ID NO: 38 - protein, 316 aa, synthetic construct
MAQTTSQVVTDIGQNAKTHTSYNTFNNEQADNMTMSLKVTFIDDPSADKQIAVINTTGSFMKANPTLSDAPVDGYPIPGASVTLRYPSQYDIAMNLQDNTSRFFHVAPTNAVEETTVTSSVDYDLGGSIFASVTPSGPSGESGATGQVTWSDSVSYKQTSYKTNLIDQTNKHVKWNVFFNGYNNQNWGIYTRDSYHALYGNQLFMYSRTYPHETDARGNLVPMNDLPTLTNSGFSPGMIAVVISEKDTEQSSIQVAYTKHADDYTLRPGFTFGTGNWVGNNIKDVDQKTFNKSFVLDWKNKKLVEKKGSAHHHHHH

SEQ ID NO: 39 - protein, 316 aa, synthetic construct
MAQTTSQVVTDIGQNAKTHTSYNTFNNEQADNMTMSLKVTFIDDPSADKQIAVINTTGSFMKANPTLSDAPVDGYPIPGASVTLRYPSQYDIAMNLQDNTSRFFHVAPTNAVEETTVTSSVDYDLGGSIFASVTPSGPSGESGATGQVTWSDSVSYDQTSYKTNLIDQTNKHVKWNVFFNGYNNQNWGIYTRDSYHALYGNQLFMYSRTYPHETDARGNLVPMNDLPTLTNSGFSPGMIAVVISEKDTEQSSIQVAYTKHADDYTLRPGFTFGTGNWVGNNIKDVDQKTFNKSFVLDWKNKKLVEKKGSAHHHHHH

SEQ ID NO: 40 - protein, 15 aa, synthetic construct
RRRRRRRRRRRRRRR

SEQ ID NO: 41 - protein, 12 aa, synthetic construct
GGGGGGGGGGGG

SEQ ID NO: 42 - protein, 425 aa, synthetic construct
MHHHHHHSSPWGAPKIEEGKLVIWINGDKGYNGLAEVGKKFEKDTGIKVTVEHPDKLEEKFPQVAATGDGPDIIFWAHDRFGGYAQSGLLAEITPDKAFQDKLYPFTWDAVRYNGKLIAYPIAVEALSLIYNKDLLPNPPKTWEEIPALDKELKAKGKSALMFNLQEPYFTWPLIAADGGYAFKYENGKYDIKDVGVDNAGAKAGLTFLVDLIKNKHMNADTDYSIAEAAFNKGETAMTINGPWAWSNIDTSKVNYGVTVLPTFKGQPSKPFVGVLSAGINAASPNKELAKEFLENYLLTDEGLEAVNKDKPLGAVALKSYEEELAKDPRIAATMENAQKGEIMPNIPQMSAFWYAVRTAVINAASGRQTVDEALKDAQTRITKHMGGGGGGGGGGGGSRRRRRRRRRRRRRRRAANDENYALAA

SEQ ID NO: 43 - protein, 766 aa, synthetic construct
MHHHHHHSSGEDIKVAVVGAMSGPVAQYGDQEFTGAEQAVADINAKGGIKGNKLQIVKYDDACDPKQAVAVANKVVNDGIKYVIGHLCSSSTQPASDIYEDEGILMITPAATAPELTARGYQLILRTTGLDSDQGPTAAKYILEKVKPQRIAIVHDKQQYGEGLARAVQDGLKKGNANVVFFDGITAGEKDFSTLVARLKKENIDFVYYGGYHPEMGQILRQARAAGLKTQFMGPEGVANVSLSNIAGESAEGLLVTKPKNYDQVPANKPIVDAIKAKKQDPSGAFVWTTYAALQSLQAGLNQSDDPAEIAKYLKANSVDTVMGPLTWDEKGDLKGFEFGVFDWHANGTATDAKVKIEEGKLVIWINGDKGYNGLAEVGKKFEKDTGIKVTVEHPDKLEEKFPQVAATGDGPDIIFWAHDRFGGYAQSGLLAEITPDKAFQDKLYPFTWDAVRYNGKLIAYPIAVEALSLIYNKDLLPNPPKTWEEIPALDKELKAKGKSALMFNLQEPYFTWPLIAADGGYAFKYENGKYDIKDVGVDNAGAKAGLTFLVDLIKNKHMNADTDYSIAEAAFNKGETAMTINGPWAWSNIDTSKVNYGVTVLPTFKGQPSKPFVGVLSAGINAASPNKELAKEFLENYLLTDEGLEAVNKDKPLGAVALKSYEEELAKDPRIAATMENAQKGEIMPNIPQMSAFWYAVRTAVINAASGRQTVDEALKDAQTRITKHMGGGGGGGGGGGGSRRRRRRRRRRRRRRRAANDENYALAA

SEQ ID NO: 44 - protein, 764 aa, synthetic construct
MHHHHHHSSGEKKSLHIYNWTDYIAPTTLKDFTKESGIDVSYDVFDSNETLEGKLVSGHSGYDIVVPSNNFLGKQIQAGAFQKLDKSKLPNWKNLDPALLKQLEVSDPGNQYAVPYLWGTNGIGYNVAKVKEVLGDQPIDSWAILFEPENMKKLAKCGVAFMDSGDEMLPAALNYLGLDPNTHDPKDYKKAEEVLTKVRPYVSYFHSSKYISDLANGNICVAFGYSGDVFQAAARAEEAGKGIDIQYVIPKEGANLWFDLMAIPADAKAADNAYAFIDYLLRPEVIAKVSDYVGYANAIPGARPLMDKSVSDSEEVYPPQAVLDKLYVSAVLPAKVLRLQTRTWTRIKTGKLEKIEEGKLVIWINGDKGYNGLAEVGKKFEKDTGIKVTVEHPDKLEEKFPQVAATGDGPDIIFWAHDRFGGYAQSGLLAEITPDKAFQDKLYPFTWDAVRYNGKLIAYPIAVEALSLIYNKDLLPNPPKTWEEIPALDKELKAKGKSALMFNLQEPYFTWPLIAADGGYAFKYENGKYDIKDVGVDNAGAKAGLTFLVDLIKNKHMNADTDYSIAEAAFNKGETAMTINGPWAWSNIDTSKVNYGVTVLPTFKGQPSKPFVGVLSAGINAASPNKELAKEFLENYLLTDEGLEAVNKDKPLGAVALKSYEEELAKDPRIAATMENAQKGEIMPNIPQMSAFWYAVRTAVINAASGRQTVDEALKDAQTRITKHMGGGGGGGGGGGGSRRRRRRRRRRRRRRRAANDENYALAA

SEQ ID NO: 45 - protein, 731 aa, synthetic construct
MHHHHHHSSGADTRIGVTIYKYDDNFMSVVRKAIEQDAKAAPDVQLLMNDSQNDQSKQNDQIDVLLAKGVKALAINLVDPAAAGTVIEKARGQNVPVVFFNKEPSRKALDSYDKAYYVGTDSKESGIIQGDLIAKHWAANQGWDLNKDGQIQFVLLKGEPGHPDAEARTTYVIKELNDKGIKTEQLQLDTAMWDTAQAKDKMDAWLSGPNANKIEVVIANNDAMAMGAVEALKAHNKSSIPVFGVDALPEALALVKSGALAGTVLNDANNQAKATFDLAKNLADGKGAADGTNWKIDNKVVRVPYVGVDKDNLAEFSKKGKIEEGKLVIWINGDKGYNGLAEVGKKFEKDTGIKVTVEHPDKLEEKFPQVAATGDGPDIIFWAHDRFGGYAQSGLLAEITPDKAFQDKLYPFTWDAVRYNGKLIAYPIAVEALSLIYNKDLLPNPPKTWEEIPALDKELKAKGKSALMFNLQEPYFTWPLIAADGGYAFKYENGKYDIKDVGVDNAGAKAGLTFLVDLIKNKHMNADTDYSIAEAAFNKGETAMTINGPWAWSNIDTSKVNYGVTVLPTFKGQPSKPFVGVLSAGINAASPNKELAKEFLENYLLTDEGLEAVNKDKPLGAVALKSYEEELAKDPRIAATMENAQKGEIMPNIPQMSAFWYAVRTAVINAASGRQTVDEALKDAQTRITKHMGGGGGGGGGGGGSRRRRRRRRRRRRRRRAANDENYALAA

SEQ ID NO: 46 - protein, 804 aa, synthetic construct
MGSSHHHHHHSSGLVPRGSHNKIEEGKLVIWINGDKGYNGLAEVGKKFEEDTGIKVTVEHPDKLEEKFPQVAATGDGPDIIFWAHDRFGGYAQSGLLAEITPDKAFQDKLYPFTWDAVRYNGKLIAYPIAVEALSLIYNKDLLPNPPKTWEEIPALDKELKAKGKSALMFNLQEPYFTWPLIAADGGYAFKYENGKYDIKDVGVDNAGAKAGLTFLVDLIKNKHMNADTDYSIAEAAFNKGETAMTINGPWAWSNIDTSKVNYGVTVLPTFKGQPSKPFVGVLSAGINAASPNKELAKEFLENYLLTDEGLEAVNKDKPLGAVALKSYEEELAKDPRIAATMENAQKGEIMPNIPQMSAFWYAVRTAVINAASGRQTVDEALKDAQTRITKGAPKIEEGKLVIWINGDKGYNGLAEVGKKFEKDTGIKVTVEHPDKLEEKFPQVAATGDGPDIIFWAHDRFGGYAQSGLLAEITPDKAFQDKLYPFTWDAVRYNGKLIAYPIAVEALSLIYNKDLLPNPPKTWEEIPALDKELKAKGKSALMFNLQEPYFTWPLIAADGGYAFKYENGKYDIKDVGVDNAGAKAGLTFLVDLIKNKHMNADTDYSIAEAAFNKGETAMTINGPWAWSNIDTSKVNYGVTVLPTFKGQPSKPFVGVLSAGINAASPNKELAKEFLENYLLTDEGLEAVNKDKPLGAVALKSYEEELAKDPRIAATMENAQKGEIMPNIPQMSAFWYAVRTAVINAASGRQTVDEALKDAQTRITKHMGGGGGGGGGGGGSRRRRRRRRRRRRRRRAANDENYALA

SEQ ID NO: 47 - protein, 273 aa, synthetic construct
MGHHHHHHSSASKGEELFTGVVPILVELDGDVNGHKFSVSGEGEGDATYGKLTLKFICTTGKLPVPWPTLVTTFSYGVQCFSRYPDHMKRHDFFKSAMPEGYVQERTIFFKDDGNYKTRAEVKFEGDTLVNRIELKGIDFKEDGNILGHKLEYNYNSHNVYIMADKQKNGIKVNFKIRHNIEDGSVQLADHYQQNTPIGDGPVLLPDNHYLSTQSALSKDPNEKRDHMVLLEFVTAAGIGGGGGGGGGGGGSRRRRRRRRRRAANDENYALAA

SEQ ID NO: 48 - protein, 278 aa, synthetic construct
MKHHHHHHGVSKGEEDNMASLPATHELHIFGSINGVDFDMVGQGTGNPNDGYEELNLKSTKGDLQFSPWILVPHIGYGFHQYLPYPDGMSPFQAAMVDGSGYQVHRTMQFEDGASLTVNYRYTYEGSHIKGEAQVKGTGFPADGPVMTNSLTAADWCRSKKTYPNDKTIISTFKWSYTTGNGKRYRSTARTTYTFAKPMAANYLKNQPMYVFRKTELKHSKTELNFKEWQKAFTDVMGMDELYKGGSGSGDYMERWYRYYNEFSGGVAANDENYALAA

SEQ ID NO: 49 - protein, 300 aa, synthetic construct
MKHHHHHHGVSKGEEDNMASLPATHELHIFGSINGVDFDMVGQGTGNPNDGYEELNLKSTKGDLQFSPWILVPHIGYGFHQYLPYPDGMSPFQAAMVDGSGYQVHRTMQFEDGASLTVNYRYTYEGSHIKGEAQVKGTGFPADGPVMTNSLTAADWCRSKKTYPNDKTIISTFKWSYTTGNGKRYRSTARTTYTFAKPMAANYLKNQPMYVFRKTELKHSKTELNFKEWQKAFTDVMGMDELYKGGSGSGDELAQLERELMKLKAQGVDSDELEALARKLAMLARSGGVAANDENYALAA

SEQ ID NO: 50 - protein, 279 aa, synthetic construct
MKHHHHHHGVSKGEEDNMASLPATHELHIFGSINGVDFDMVGQGTGNPNDGYEELNLKSTKGDLQFSPWILVPHIGYGFHQYLPYPDGMSPFQAAMVDGSGYQVHRTMQFEDGASLTVNYRYTYEGSHIKGEAQVKGTGFPADGPVMTNSLTAADWCRSKKTYPNDKTIISTFKWSYTTGNGKRYRSTARTTYTFAKPMAANYLKNQPMYVFRKTELKHSKTELNFKEWQKAFTDVMGMDELYKGGSGSGRGKITVNGKTYEGRSGGVAANDENYALAA

SEQ ID NO: 51 - protein, 584 aa, synthetic construct
MGSSHHHHHHGSGLVPRGSAGEVSRISYEDIGGLSEQLGKIREMIELPLKHPELFERLGITPPKGVILYGPPGTGKTLIARAVANESGANFLSINGPEIMSKYYGQSEQKLREIFSKAEETAPSIIFIDEIDSIAPKREEVQGEVERRVVAQLLTLMDGMKERGHVIVIGATNRIDAIDPALRRPGRFDREIEIGVPDRNGRKEILMIHTRNMPLGMSEEEKNKFLEEMADYTYGFVGADLAALVRESAMNALRRYLPEIDLDKPIPTEILEKMVVTEDDFKNALKSIEPSSLREVMVEVPNVHWDDIGGLEDVKREIKETVELPLLKPDVFKRLGIRPSKGFLLYGPPGVGKTLLAKAVATESNANFISIKGPEVLSKWVGESEKAIREIFKKAKQVAPAIVFLDEIDSIAPRRGTTSDSGVTERIVNQLLTSLDGIEVMNGVVVIGATNRPDIMDPALLRAGRFDKLIYIPPPDKEARLSILKVHTKNMPLAPDVDLNDIAQRTEGYVGADLENLCREAGMNAYRENPDATSVSQKNFLDALKTIRPSVDEEVIKFYRTLSETMSKSVSERRKQLQDQGLYL

SEQ ID NO: 52 - protein, 392 aa, synthetic construct
MGCHHHHHHSSGLVPRGSHNKIEEGKLVIWINGDKGYNGLAEVGKKFEEDTGIKVTVEHPDKLEEKFPQVAATGDGPDIIFWAHDRFGGYAQSGLLAEITPDKAFQDKLYPFTWDAVRYNGKLIAYPIAVEALSLIYNKDLLPNPPKTWEEIPALDKELKAKGKSALMFNLQEPYFTWPLIAADGGYAFKYENGKYDIKDVGVDNAGAKAGLTFLVDLIKNKHMNADTDYSIAEAAFNKGETAMTINGPWAWSNIDTSKVNYGVTVLPTFKGQPSKPFVGVLSAGINAASPNKELAKEFLENYLLTDEGLEAVNKDKPLGAVALKSYEEELAKDPRIAATMENAQKGEIMPNIPQMSAFWYAVRTAVINAASGRQTVDEALKDAQTRITKSS

SEQ ID NO: 53 - protein, 394 aa, synthetic construct
MGSSHHHHHHSSGLVPRGSHNKIEEGKLVIWINGDKGYNGLAEVGKKFEEDTGIKVTVEHPDKLEEKFPQVAATGDGPDIIFWAHDRFGGYAQSGLLAEITPDKAFQDKLYPFTWDAVRYNGKLIAYPIAVEALSLIYNKDLLPNPPKTWEEIPALDKELKAKGKSALMFNLQEPYFTWPLIAADGGYAFKYENGKYDIKDVGVDNAGAKAGLTFLVDLIKNKHMNADTDYSIAEAAFNKGETAMTINGPWAWSNIDTSKVNYGVTVLPTFKGQPSKPFVGVLSAGINAASPNKELAKEFLENYLLTDEGLEAVNKDKPLGAVALKSYEEELAKDPRIAATMENAQKGEIMPNIPQMSAFWYAVRTAVINAASGRQTVDEALKDAQTRITKSSC

SEQ ID NO: 54 - protein, 42 aa, synthetic construct
GGGGGGGGGGGGRRRRRRRRRRRRRRRSGGVAANDENYALAA

SEQ ID NO: 55 - protein, 293 aa, synthetic construct
ADSDINIKTGTTDIGSNTTVKTGDLVTYDKENGMHKKVFYSFIDDKNHNKKLLVIRTKGTIAGQYRVYSEEGANKSGLAWPSAFKVQLQLPDNEVAQISDYYPRNSIDTKEYMSTLTYDFDGDVDGDDTGKIGGCIGANVSIGHTLKYVQPDFKTILESPTDKKVGWKVIFNNMVNQNWGPYDRDSWNPVYGNQLFMKTRNGSMKAADNFLDPNKASSLLSSGFSPDFATVITMDRKASKQQTNIDVIYERVRDDYQLHWTSTNWKGTNTKDKWTDRSSERYKIDWEKEEMTN

SEQ ID NO: 56 - protein, 262 aa, synthetic construct
CLTAPPKEAARPTLMPRAQSYKDLTHLPAPTGKIFVSVYNIQDETGQFKPYPASNDSTAVPQSATAMLVTALKDSRWFIPLERQGLQNLLNERKIIRAAQENGTVAINNRIPLQSLTAANIMVEGSIIGYESNVKSGGVGARYFGIGADTQYQLDQIAVNLRVVNVSTGEILSSVNTSKTILSYEVQAGVFRFIDYQRLLEGEVGYTSNEPVMLCLMSAIETGVIFLINDGIDRGLWDLQNKAERQNDILVKYRHMSVPPES

SEQ ID NO: 57 - protein, 119 aa, synthetic construct
GTMTFQFRNPNFGGNPNNGAFLLNSAQAQNSYKDPSYNDDFGIETPSALDNFTQAIQSQILGGLLSNINTGKPGRMVTNDYIVDIANRDGQLQLNVTDRKTGQTSTIQVSGLQNNSTDF

SEQ ID NO: 58 - protein, 9 aa, synthetic construct
GGGGGGGGG